European Patent Application EP 4 130 046 A1, published February 8, 2023. Title: Platform for Constructing Multispecific Antibody. Applicant: BIOTHEUS INC. The sequence listing filed with the application follows.

SEQUENCE LISTING (60 sequences)

SEQ ID NO: 1 - protein, 480 aa, Artificial Sequence
  Amino acid sequence of Peptide #1 of Bi-70-71
EVQLVESGGGLVQPGNSLRLSCAASGFTFSSFGMSWVRQAPGKGLEWVSSISGSGSDTLYADSVKGRFTISRDNAKTTLYLQMNSLRPEDTAVYYCTIGGSLSRSSQGTLVTVSSGGGGSGGGGSGQVQLVQSGVEVKKPGASVKVSCKASGYTFTNYYMYWVRQAPGQGLEWMGGINPSNGGTNFNEKFKNRVTLTTDSSTTTAYMELKSLQFDDTAVYYCARRDYRFDMGFDYWGQGTTVTVSSASTKGPSVFPLAPSSKSTSGGTAALGCLVKDYFPEPVTVSWNSGALTSGVHTFPAVLQSSGLYSLSSVVTVPSSSLGTQTYICNVNHKPSNTKVDKKVEPKSCGGGGSGGGGSGQVQLQESGGGLVQAGGSLRLSCVASGSIFSIGTMGWYRQAPGKQRDLVALVTIDGSTNYPDSVKGRFTISRDNVKNTVDLQMNSLEPEDTAVYYCNANIRTGWSSVRTYWGQGTQVTVSS

SEQ ID NO: 2 - protein, 120 aa, Artificial Sequence [sequence omitted]

SEQ ID NO: 3 - protein, 103 aa, Homo sapiens
ASTKGPSVFPLAPSSKSTSGGTAALGCLVKDYFPEPVTVSWNSGALTSGVHTFPAVLQSSGLYSLSSVVTVPSSSLGTQTYICNVNHKPSNTKVDKKVEPKSC

SEQ ID NO: 4 - protein, 11 aa, Artificial Sequence
  Linker sequence
GGGGSGGGGSG

SEQ ID NO: 5 - protein, 115 aa, Artificial Sequence [sequence omitted]

SEQ ID NO: 6 - protein, 120 aa, Artificial Sequence
  Amino acid sequence of Anti-TIGIT nanobody
QVQLQESGGGLVQAGGSLRLSCVASGSIFSIGTMGWYRQAPGKQRDLVALVTIDGSTNYPDSVKGRFTISRDNVKNTVDLQMNSLEPEDTAVYYCNANIRTGWSSVRTYWGQGTQVTVSS

SEQ ID NO: 7 - protein, 218 aa, Artificial Sequence
  Amino acid sequence of Peptide #2 of Bi-70-71
EIVLTQSPATLSLSPGERATLSCRASKGVSTSGYSYLHWYQQKPGQAPRLLIYLASYLESGVPARFSGSGSGTDFTLTISSLEPEDFAVYYCQHSRDLPLTFGGGTKVEIKRTVAAPSVFIFPPSDEQLKSGTASVVCLLNNFYPREAKVQWKVDNALQSGNSQESVTEQDSKDSTYSLSSTLTLSKADYEKHKVYACEVTHQGLSSPVTKSFNRGEC

SEQ ID NO: 8 - protein, 111 aa, Artificial Sequence [sequence omitted]

SEQ ID NO: 9 - protein, 107 aa, Homo sapiens [sequence omitted]

SEQ ID NO: 10 - protein, 223 aa, Artificial Sequence
  Amino acid sequence of Peptide #1 of Bi-72-73
QVQLVQSGVEVKKPGASVKVSCKASGYTFTNYYMYWVRQAPGQGLEWMGGINPSNGGTNFNEKFKNRVTLTTDSSTTTAYMELKSLQFDDTAVYYCARRDYRFDMGFDYWGQGTTVTVSSASTKGPSVFPLAPSSKSTSGGTAALGCLVKDYFPEPVTVSWNSGALTSGVHTFPAVLQSSGLYSLSSVVTVPSSSLGTQTYICNVNHKPSNTKVDKKVEPKSC

SEQ ID NO: 11 - protein, 475 aa, Artificial Sequence
  Amino acid sequence of Peptide #2 of Bi-72-73
EVQLVESGGGLVQPGNSLRLSCAASGFTFSSFGMSWVRQAPGKGLEWVSSISGSGSDTLYADSVKGRFTISRDNAKTTLYLQMNSLRPEDTAVYYCTIGGSLSRSSQGTLVTVSSGGGGSGGGGSGEIVLTQSPATLSLSPGERATLSCRASKGVSTSGYSYLHWYQQKPGQAPRLLIYLASYLESGVPARFSGSGSGTDFTLTISSLEPEDFAVYYCQHSRDLPLTFGGGTKVEIKRTVAAPSVFIFPPSDEQLKSGTASVVCLLNNFYPREAKVQWKVDNALQSGNSQESVTEQDSKDSTYSLSSTLTLSKADYEKHKVYACEVTHQGLSSPVTKSFNRGECGGGGSGGGGSGQVQLQESGGGLVQAGGSLRLSCVASGSIFSIGTMGWYRQAPGKQRDLVALVTIDGSTNYPDSVKGRFTISRDNVKNTVDLQMNSLEPEDTAVYYCNANIRTGWSSVRTYWGQGTQVTVSS

SEQ ID NO: 12 - protein, 478 aa, Artificial Sequence
  Amino acid sequence of Peptide #1 of Bi-74-76
EVQLVESGGGLVQPGNSLRLSCAASGFTFSSFGMSWVRQAPGKGLEWVSSISGSGSDTLYADSVKGRFTISRDNAKTTLYLQMNSLRPEDTAVYYCTIGGSLSRSSQGTLVTVSSGGGGSGGGGSGEVQLVESGGGLVQPGGSLRLSCAASGYTFTNYGMNWVRQAPGKGLEWVGWINTYTGEPTYAADFKRRFTFSLDTSKSTAYLQMNSLRAEDTAVYYCAKYPHYYGSSHWYFDVWGQGTLVTVSSASTKGPSVFPLAPSSKSTSGGTAALGCLVKDYFPEPVTVSWNSGALTSGVHTFPAVLQSSGLYSLSSVVTVPSSSLGTQTYICNVNHKPSNTKVDKKVEPKSCGGGGSGGGGSGEVQLQESGGGLVQPGGSLRLSCAASGFTFSSYWMYWLRQAPGKGLEWVSSINSDSSSTYYRDSVKGRFTISRDNAKNTLYLQMNSLKSEDTAVYYCAKDPGGYAKGQGTQVTVSS

SEQ ID NO: 13 - protein, 226 aa, Artificial Sequence
  Amino acid sequence of VH chain of anti-VEGF antibody
EVQLVESGGGLVQPGGSLRLSCAASGYTFTNYGMNWVRQAPGKGLEWVGWINTYTGEPTYAADFKRRFTFSLDTSKSTAYLQMNSLRAEDTAVYYCAKYPHYYGSSHWYFDVWGQGTLVTVSSASTKGPSVFPLAPSSKSTSGGTAALGCLVKDYFPEPVTVSWNSGALTSGVHTFPAVLQSSGLYSLSSVVTVPSSSLGTQTYICNVNHKPSNTKVDKKVEPKSC

SEQ ID NO: 14 - protein, 115 aa, Artificial Sequence
  Amino acid sequence of Anti-PD-L1 nanobody
EVQLQESGGGLVQPGGSLRLSCAASGFTFSSYWMYWLRQAPGKGLEWVSSINSDSSSTYYRDSVKGRFTISRDNAKNTLYLQMNSLKSEDTAVYYCAKDPGGYAKGQGTQVTVSS

SEQ ID NO: 15 - protein, 340 aa, Artificial Sequence
  Amino acid sequence of Peptide #2 of Bi-74-76
DIQMTQSPSSLSASVGDRVTITCSASQDISNYLNWYQQKPGKAPKVLIYFTSSLHSGVPSRFSGSGSGTDFTLTISSLQPEDFATYYCQQYSTVPWTFGQGTKVEIKRTVAAPSVFIFPPSDEQLKSGTASVVCLLNNFYPREAKVQWKVDNALQSGNSQESVTEQDSKDSTYSLSSTLTLSKADYEKHKVYACEVTHQGLSSPVTKSFNRGECGGGGSGGGGSGEVQLQESGGGLVQPGGSLRLSCAASGFTFSSYWMYWLRQAPGKGLEWVSSINSDSSSTYYRDSVKGRFTISRDNAKNTLYLQMNSLKSEDTAVYYCAKDPGGYAKGQGTQVTVSS

SEQ ID NO: 16 - protein, 107 aa, Artificial Sequence [sequence omitted]

SEQ ID NO: 17 - protein, 344 aa, Artificial Sequence
  Amino acid sequence of Peptide #1 of Bi-78-79, Bi-79-83, Bi-79-86
EVQLQESGGGLVQPGGSLRLSCAASGFTFSSYWMYWLRQAPGKGLEWVSSINSDSSSTYYRDSVKGRFTISRDNAKNTLYLQMNSLKSEDTAVYYCAKDPGGYAKGQGTQVTVSSASTKGPSVFPLAPSSKSTSGGTAALGCLVKDYFPEPVTVSWNSGALTSGVHTFPAVLQSSGLYSLSSVVTVPSSSLGTQTYICNVNHKPSNTKVDKKVEPKSCGGGGSGGGGSGEVQLVESGGGLVQPGNSLRLSCAASGFTFSSFGMSWVRQAPGKGLEWVSSISGSGSDTLYADSVKGRFTISRDNAKTTLYLQMNSLRPEDTAVYYCTIGGSLSRSSQGTLVTVSS

SEQ ID NO: 18 - protein, 223 aa, Artificial Sequence
  Amino acid sequence of Peptide #2 of Bi-78-79, Bi-79-80
QVQLQESGGGLVQAGDSLRLSCIGSRRTFTMAWFRQAPGKEREFVAGIWGPADHTIYANSVKGRFACSRDDSTNTIFLQMNSLELEDTALYLCAAADSSGDDFEYWGQGTQVTVSSRTVAAPSVFIFPPSDEQLKSGTASVVCLLNNFYPREAKVQWKVDNALQSGNSQESVTEQDSKDSTYSLSSTLTLSKADYEKHKVYACEVTHQGLSSPVTKSFNRGEC

SEQ ID NO: 19 - protein, 116 aa, Artificial Sequence
  Amino acid sequence of Anti-PD-L2 nanobody
QVQLQESGGGLVQAGDSLRLSCIGSRRTFTMAWFRQAPGKEREFVAGIWGPADHTIYANSVKGRFACSRDDSTNTIFLQMNSLELEDTALYLCAAADSSGDDFEYWGQGTQVTVSS

SEQ ID NO: 20 - protein, 338 aa, Artificial Sequence
  Amino acid sequence of Peptide #1 of Bi-78-80
EVQLQESGGGLVQPGGSLRLSCAASGFTFSSYWMYWLRQAPGKGLEWVSSINSDSSSTYYRDSVKGRFTISRDNAKNTLYLQMNSLKSEDTAVYYCAKDPGGYAKGQGTQVTVSSASTKGPSVFPLAPSSKSTSGGTAALGCLVKDYFPEPVTVSWNSGALTSGVHTFPAVLQSSGLYSLSSVVTVPSSSLGTQTYICNVNHKPSNTKVDKKVEPKSCDKTHTEVQLVESGGGLVQPGNSLRLSCAASGFTFSSFGMSWVRQAPGKGLEWVSSISGSGSDTLYADSVKGRFTISRDNAKTTLYLQMNSLRPEDTAVYYCTIGGSLSRSSQGTLVTVSS

SEQ ID NO: 21 - protein, 5 aa, Artificial Sequence
  Linker sequence of Bi-78-80
DKTHT

SEQ ID NO: 22 - protein, 355 aa, Artificial Sequence
  Amino acid sequence of Peptide #1 of Bi-81-82
EVQLQESGGGLVQPGGSLRLSCAASGFTFSSYWMYWLRQAPGKGLEWVSSINSDSSSTYYRDSVKGRFTISRDNAKNTLYLQMNSLKSEDTAVYYCAKDPGGYAKGQGTQVTVSSGGGGSGGGGSGASTKGPSVFPLAPSSKSTSGGTAALGCLVKDYFPEPVTVSWNSGALTSGVHTFPAVLQSSGLYSLSSVVTVPSSSLGTQTYICNVNHKPSNTKVDKKVEPKSCGGGGSGGGGSGEVQLVESGGGLVQPGNSLRLSCAASGFTFSSFGMSWVRQAPGKGLEWVSSISGSGSDTLYADSVKGRFTISRDNAKTTLYLQMNSLRPEDTAVYYCTIGGSLSRSSQGTLVTVSS

SEQ ID NO: 23 - protein, 234 aa, Artificial Sequence
  Amino acid sequence of Peptide #2 of Bi-81-82
QVQLQESGGGLVQAGDSLRLSCIGSRRTFTMAWFRQAPGKEREFVAGIWGPADHTIYANSVKGRFACSRDDSTNTIFLQMNSLELEDTALYLCAAADSSGDDFEYWGQGTQVTVSSGGGGSGGGGSGRTVAAPSVFIFPPSDEQLKSGTASVVCLLNNFYPREAKVQWKVDNALQSGNSQESVTEQDSKDSTYSLSSTLTLSKADYEKHKVYACEVTHQGLSSPVTKSFNRGEC

SEQ ID NO: 24 - protein, 354 aa, Artificial Sequence
  Amino acid sequence of Peptide #2 of Bi-79-83
QVQLQESGGGLVQAGDSLRLSCIGSRRTFTMAWFRQAPGKEREFVAGIWGPADHTIYANSVKGRFACSRDDSTNTIFLQMNSLELEDTALYLCAAADSSGDDFEYWGQGTQVTVSSRTVAAPSVFIFPPSDEQLKSGTASVVCLLNNFYPREAKVQWKVDNALQSGNSQESVTEQDSKDSTYSLSSTLTLSKADYEKHKVYACEVTHQGLSSPVTKSFNRGECGGGGSGGGGSGQVQLQESGGGLVQAGGSLRLSCVASGSIFSIGTMGWYRQAPGKQRDLVALVTIDGSTNYPDSVKGRFTISRDNVKNTVDLQMNSLEPEDTAVYYCNANIRTGWSSVRTYWGQGTQVTVSS

SEQ ID NO: 25 - protein, 223 aa, Artificial Sequence
  Amino acid sequence of Peptide #2 of Bi-79-86
QVQLVESGGGLVPPGESLRLSCAASGAIFRINTGAWYRQAPGKQRELVASLTTYGKTTYADFVKGRFTISRDDAKNTVYLQMNSLKPEDTAIYYCHIGPEPRYGYWGQGTQVTVSSRTVAAPSVFIFPPSDEQLKSGTASVVCLLNNFYPREAKVQWKVDNALQSGNSQESVTEQDSKDSTYSLSSTLTLSKADYEKHKVYACEVTHQGLSSPVTKSFNRGEC

SEQ ID NO: 26 - protein, 116 aa, Artificial Sequence
  Amino acid sequence of Anti-41BB nanobody
QVQLVESGGGLVPPGESLRLSCAASGAIFRINTGAWYRQAPGKQRELVASLTTYGKTTYADFVKGRFTISRDDAKNTVYLQMNSLKPEDTAIYYCHIGPEPRYGYWGQGTQVTVSS

SEQ ID NO: 27 - protein, 453 aa, Artificial Sequence
  Amino acid sequence of Peptide #1 of Bi-203-204
QVQLVESGGGLVKPGGSLRLSCAASGHTFIIYAIGWFRQAPGKGLEFVATINWSGSMTNYADSVKGRFTISRDNAKNTVYLQMNSLKPDDTAVYYCAAYVGATISTAHSRYDYWGQGTLVTVSSASTKGPSVFPLAPSSKSTSGGTAALGCLVKDYFPEPVTVSWNSGALTSGVHTFPAVLQSSGLYSLSSVVTVPSSSLGTQTYICNVNHKPSNTKVDKKVEPKSCDKTHTCPPCPAPEAAGGPSVFLFPPKPKDTLMISRTPEVTCVVVDVSHEDPEVKFNWYVDGVEVHNAKTKPREEQYNSTYRVVSVLTVLHQDWLNGKEYKCKVSNKALPAPIEKTISKAKGQPREPQVYTLPPSREEMTKNQVSLTCLVKGFYPSDIAVEWESNGQPENNYKTTPPVLDSDGSFFLYSKLTVDKSRWQQGNVFSCSVMHEALHNHYTQKSLSLSPG

SEQ ID NO: 28 - protein, 124 aa, Artificial Sequence
  Amino acid sequence of Anti-PD-L1 nanobody
QVQLVESGGGLVKPGGSLRLSCAASGHTFIIYAIGWFRQAPGKGLEFVATINWSGSMTNYADSVKGRFTISRDNAKNTVYLQMNSLKPDDTAVYYCAAYVGATISTAHSRYDYWGQGTLVTVSS

SEQ ID NO: 29 - protein, 226 aa, Artificial Sequence
  Amino acid sequence of LALA mutant Fc of human IgG1
DKTHTCPPCPAPEAAGGPSVFLFPPKPKDTLMISRTPEVTCVVVDVSHEDPEVKFNWYVDGVEVHNAKTKPREEQYNSTYRVVSVLTVLHQDWLNGKEYKCKVSNKALPAPIEKTISKAKGQPREPQVYTLPPSREEMTKNQVSLTCLVKGFYPSDIAVEWESNGQPENNYKTTPPVLDSDGSFFLYSKLTVDKSRWQQGNVFSCSVMHEALHNHYTQKSLSLSPG

SEQ ID NO: 30 - protein, 226 aa, Artificial Sequence
  Amino acid sequence of Peptide #2 of Bi-203-204
EVQLVESGGGLVQPGGSLRLSCAASGRTFSSMTIGWFRQAPGKGLEFVSGIGWTSGLTVYADSVKGRFTISRDNAKNSMYLQMNSLRAEDTAVYYCAADSMNRGQFDYWGQGTLVTVSSRTVAAPSVFIFPPSDEQLKSGTASVVCLLNNFYPREAKVQWKVDNALQSGNSQESVTEQDSKDSTYSLSSTLTLSKADYEKHKVYACEVTHQGLSSPVTKSFNRGEC

SEQ ID NO: 31 - protein, 119 aa, Artificial Sequence
  Amino acid sequence of Anti-PD-L2 nanobody
EVQLVESGGGLVQPGGSLRLSCAASGRTFSSMTIGWFRQAPGKGLEFVSGIGWTSGLTVYADSVKGRFTISRDNAKNSMYLQMNSLRAEDTAVYYCAADSMNRGQFDYWGQGTLVTVSS

SEQ ID NO: 32 - DNA, 1443 bp, Artificial Sequence
  Nucleotide sequence of Peptide #1 of Bi-70-71
gaggtgcagctggtcgaaagcggcggcggactggtgcaacccggcaattctctgaggctgagctgtgccgctagcggcttcaccttcagcagcttcggcatgagctgggtcagacaagcccccggcaagggactggagtgggtgagctccatcagcggcagcggaagcgatactctgtacgccgacagcgtgaagggaaggttcaccatctctagggacaacgccaagaccactctgtatctgcagatgaactctctgaggcccgaggataccgccgtgtactactgcaccatcggcggatctctgagcagaagcagccaaggcactctggtcaccgtcagcagcggcggaggcgggagcggaggcggaggctccggacaagtgcagctggtgcagagcggcgtggaggtgaagaaacccggcgctagcgtgaaggtgagctgcaaggccagcggctacaccttcaccaactactacatgtattgggtgaggcaagcccccggccaaggactggagtggatgggcggcatcaatcccagcaacggcggcaccaacttcaacgagaagttcaagaatagggtgaccctcaccactgatagcagcaccaccaccgcctacatggagctgaagagcctccagttcgacgataccgccgtctactactgcgccagaagggactataggttcgacatgggcttcgactattggggccaaggcaccactgtgaccgtgagcagcgccagcactaagggccctagcgtcttccctctggcccctagcagcaagagcaccagcggaggaactgctgctctgggctgtctggtgaaggactacttccccgagcccgtgaccgtgagctggaacagcggcgctctgactagcggcgtgcacactttccccgccgtgctgcagagcagcggactgtactctctgagcagcgtggtgactgtccccagcagctctctgggcactcagacctacatctgcaacgtcaaccacaagcccagcaacaccaaggtcgacaagaaggtcgagcctaagagctgcggcggaggcgggagcggaggcggaggctccggacaagtgcagctgcaagagagcggaggaggactggtccaagctggaggctctctgagactgagctgcgtggccagcggcagcatcttctccatcggcaccatgggctggtacagacaagcccccggcaagcagagggatctggtggctctggtgaccatcgatggcagcaccaattaccccgatagcgtgaagggaaggttcaccatctctagggacaacgtgaagaacaccgtggatctgcagatgaactctctggagcccgaggataccgccgtgtactactgcaatgccaacattaggaccggctggagcagcgtgaggacttactggggccaaggcacccaagtgactgtgtccagctga

SEQ ID NO: 33 - DNA, 360 bp, Artificial Sequence
  Nucleotide sequence of VH chain of anti-PD-1 antibody
caagtgcagctggtgcagagcggcgtggaggtgaagaaacccggcgctagcgtgaaggtgagctgcaaggccagcggctacaccttcaccaactactacatgtattgggtgaggcaagcccccggccaaggactggagtggatgggcggcatcaatcccagcaacggcggcaccaacttcaacgagaagttcaagaatagggtgaccctcaccactgatagcagcaccaccaccgcctacatggagctgaagagcctccagttcgacgataccgccgtctactactgcgccagaagggactataggttcgacatgggcttcgactattggggccaaggcaccactgtgaccgtgagcagc

SEQ ID NO: 34 - DNA, 309 bp, Homo sapiens
gccagcactaagggccctagcgtcttccctctggcccctagcagcaagagcaccagcggaggaactgctgctctgggctgtctggtgaaggactacttccccgagcccgtgaccgtgagctggaacagcggcgctctgactagcggcgtgcacactttccccgccgtgctgcagagcagcggactgtactctctgagcagcgtggtgactgtccccagcagctctctgggcactcagacctacatctgcaacgtcaaccacaagcccagcaacaccaaggtcgacaagaaggtcgagcctaagagctgc

SEQ ID NO: 35 - DNA, 345 bp, Artificial Sequence
  Nucleotide sequence of Anti-human serum albumin nanobody
gaggtgcagctggtcgaaagcggcggcggactggtgcaacccggcaattctctgaggctgagctgtgccgctagcggcttcaccttcagcagcttcggcatgagctgggtcagacaagcccccggcaagggactggagtgggtgagctccatcagcggcagcggaagcgatactctgtacgccgacagcgtgaagggaaggttcaccatctctagggacaacgccaagaccactctgtatctgcagatgaactctctgaggcccgaggataccgccgtgtactactgcaccatcggcggatctctgagcagaagcagccaaggcactctggtcaccgtcagcagc

SEQ ID NO: 36 - DNA, 363 bp, Artificial Sequence
  Nucleotide sequence of Anti-TIGIT nanobody
caagtgcagctgcaagagagcggaggaggactggtccaagctggaggctctctgagactgagctgcgtggccagcggcagcatcttctccatcggcaccatgggctggtacagacaagcccccggcaagcagagggatctggtggctctggtgaccatcgatggcagcaccaattaccccgatagcgtgaagggaaggttcaccatctctagggacaacgtgaagaacaccgtggatctgcagatgaactctctggagcccgaggataccgccgtgtactactgcaatgccaacattaggaccggctggagcagcgtgaggacttactggggccaaggcacccaagtgactgtgtccagctga

SEQ ID NO: 37 - DNA, 654 bp, Artificial Sequence
  Nucleotide sequence of Peptide #2 of Bi-70-71
gagatcgtgctgacccagagccccgctactctgtctctgagccccggcgagagagccactctgagctgtagagccagcaaaggcgtcagcaccagcggctacagctatctgcactggtaccagcagaagcccggccaagcccccagactgctcatctatctggctagctatctggagagcggcgtgcccgccagattctccggaagcggcagcggcaccgactttaccctcaccatcagctctctggagcccgaggacttcgccgtgtactactgccagcactctagggatctgcctctgacctttggcggcggcactaaggtggagatcaagaggaccgtcgccgcccccagcgtgttcatcttccctcctagcgatgagcagctgaagagcggcactgccagcgtcgtctgtctgctgaacaatttctaccctagggaggccaaggtgcagtggaaggtggataacgctctgcagagcggcaacagccaagagtccgtcaccgagcaagatagcaaagatagcacctacagcctcagcagcactctgactctgtccaaggccgattacgagaagcacaaggtgtacgcttgcgaggtgactcaccaaggactgagcagccccgtgaccaagagcttcaataggggcgagtgt

SEQ ID NO: 38 - DNA, 333 bp, Artificial Sequence
  Nucleotide sequence of VL chain of anti-PD-1 antibody
gagatcgtgctgacccagagccccgctactctgtctctgagccccggcgagagagccactctgagctgtagagccagcaaaggcgtcagcaccagcggctacagctatctgcactggtaccagcagaagcccggccaagcccccagactgctcatctatctggctagctatctggagagcggcgtgcccgccagattctccggaagcggcagcggcaccgactttaccctcaccatcagctctctggagcccgaggacttcgccgtgtactactgccagcactctagggatctgcctctgacctttggcggcggcactaaggtggagatcaag

SEQ ID NO: 39 - DNA, 321 bp, Homo sapiens
aggaccgtcgccgcccccagcgtgttcatcttccctcctagcgatgagcagctgaagagcggcactgccagcgtcgtctgtctgctgaacaatttctaccctagggaggccaaggtgcagtggaaggtggataacgctctgcagagcggcaacagccaagagtccgtcaccgagcaagatagcaaagatagcacctacagcctcagcagcactctgactctgtccaaggccgattacgagaagcacaaggtgtacgcttgcgaggtgactcaccaaggactgagcagccccgtgaccaagagcttcaataggggcgagtgt

SEQ ID NO: 40 - DNA, 669 bp, Artificial Sequence
  Nucleotide sequence of Peptide #1 of Bi-72-73
caagtgcagctggtgcagagcggcgtggaggtgaagaaacccggcgctagcgtgaaggtgagctgcaaggccagcggctacaccttcaccaactactacatgtattgggtgaggcaagcccccggccaaggactggagtggatgggcggcatcaatcccagcaacggcggcaccaacttcaacgagaagttcaagaatagggtgaccctcaccactgatagcagcaccaccaccgcctacatggagctgaagagcctccagttcgacgataccgccgtctactactgcgccagaagggactataggttcgacatgggcttcgactattggggccaaggcaccactgtgaccgtgagcagcgccagcactaagggccctagcgtcttccctctggcccctagcagcaagagcaccagcggaggaactgctgctctgggctgtctggtgaaggactacttccccgagcccgtgaccgtgagctggaacagcggcgctctgactagcggcgtgcacactttccccgccgtgctgcagagcagcggactgtactctctgagcagcgtggtgactgtccccagcagctctctgggcactcagacctacatctgcaacgtcaaccacaagcccagcaacaccaaggtcgacaagaaggtcgagcctaagagctgc

SEQ ID NO: 41 - DNA, 1425 bp, Artificial Sequence
  Nucleotide sequence of Peptide #2 of Bi-72-73
gaggtgcagctggtcgaaagcggcggcggactggtgcaacccggcaattctctgaggctgagctgtgccgctagcggcttcaccttcagcagcttcggcatgagctgggtcagacaagcccccggcaagggactggagtgggtgagctccatcagcggcagcggaagcgatactctgtacgccgacagcgtgaagggaaggttcaccatctctagggacaacgccaagaccactctgtatctgcagatgaactctctgaggcccgaggataccgccgtgtactactgcaccatcggcggatctctgagcagaagcagccaaggcactctggtcaccgtcagcagcggcggaggcgggagcggaggcggaggctccggagagatcgtgctgacccagagccccgctactctgtctctgagccccggcgagagagccactctgagctgtagagccagcaaaggcgtcagcaccagcggctacagctatctgcactggtaccagcagaagcccggccaagcccccagactgctcatctatctggctagctatctggagagcggcgtgcccgccagattctccggaagcggcagcggcaccgactttaccctcaccatcagctctctggagcccgaggacttcgccgtgtactactgccagcactctagggatctgcctctgacctttggcggcggcactaaggtggagatcaagaggaccgtcgccgcccccagcgtgttcatcttccctcctagcgatgagcagctgaagagcggcactgccagcgtcgtctgtctgctgaacaatttctaccctagggaggccaaggtgcagtggaaggtggataacgctctgcagagcggcaacagccaagagtccgtcaccgagcaagatagcaaagatagcacctacagcctcagcagcactctgactctgtccaaggccgattacgagaagcacaaggtgtacgcttgcgaggtgactcaccaaggactgagcagccccgtgaccaagagcttcaataggggcgagtgtggcggaggcgggagcggaggcggaggctccggacaagtgcagctgcaagagagcggaggaggactggtccaagctggaggctctctgagactgagctgcgtggccagcggcagcatcttctccatcggcaccatgggctggtacagacaagcccccggcaagcagagggatctggtggctctggtgaccatcgatggcagcaccaattaccccgatagcgtgaagggaaggttcaccatctctagggacaacgtgaagaacaccgtggatctgcagatgaactctctggagcccgaggataccgccgtgtactactgcaatgccaacattaggaccggctggagcagcgtgaggacttactggggccaaggcacccaagtgactgtgtccagc

SEQ ID NO: 42 - DNA, 1437 bp, Artificial Sequence
  Nucleotide sequence of Peptide #1 of Bi-74-76
gaggtgcagctggtcgaaagcggcggcggactggtgcaacccggcaattctctgaggctgagctgtgccgctagcggcttcaccttcagcagcttcggcatgagctgggtcagacaagcccccggcaagggactggagtgggtgagctccatcagcggcagcggaagcgatactctgtacgccgacagcgtgaagggaaggttcaccatctctagggacaacgccaagaccactctgtatctgcagatgaactctctgaggcccgaggataccgccgtgtactactgcaccatcggcggatctctgagcagaagcagccaaggcactctggtcaccgtcagcagcggcggaggcgggagcggaggcggaggctccggagaggtccagctggtcgaatccggcggaggactggtccaacccggcggatctctgagactcagctgcgctgccagcggctacaccttcaccaactacggcatgaactgggtgaggcaagcccccggcaaaggactggagtgggtgggctggatcaacacctacactggcgaacccacctacgccgccgacttcaagaggagattcaccttctctctggacacctccaagagcaccgcttatctgcagatgaactctctgagggccgaggataccgccgtctactactgcgccaagtaccctcactactacggcagcagccactggtacttcgatgtgtggggccaaggcactctggtcactgtcagcagcgccagcactaagggccctagcgtcttccctctggcccctagcagcaagagcaccagcggaggaactgctgctctgggctgtctggtgaaggactacttccccgagcccgtgaccgtgagctggaacagcggcgctctgactagcggcgtgcacactttccccgccgtgctgcagagcagcggactgtactctctgagcagcgtggtgactgtccccagcagctctctgggcactcagacctacatctgcaacgtcaaccacaagcccagcaacaccaaggtcgacaagaaggtcgagcctaagagctgcggcggaggcgggagcggaggcggaggctccggagaggtccagctgcaagagagcggcggaggactggtgcaacccggcggctctctgagactcagctgtgccgccagcggcttcaccttcagcagctactggatgtactggctcagacaagcccccggcaaaggactggaatgggtgtccagcatcaacagcgacagcagcagcacctactatagggatagcgtcaagggaaggttcaccatctctagggacaacgccaagaacactctgtatctgcagatgaactctctgaagagcgaggataccgccgtgtactactgcgccaaggatcccggcggctatgctaaaggccaaggcactcaagtcactgtgagcagctga

SEQ ID NO: 43 - DNA, 678 bp, Artificial Sequence
  Nucleotide sequence of VH chain of anti-VEGF antibody
gaggtccagctggtcgaatccggcggaggactggtccaacccggcggatctctgagactcagctgcgctgccagcggctacaccttcaccaactacggcatgaactgggtgaggcaagcccccggcaaaggactggagtgggtgggctggatcaacacctacactggcgaacccacctacgccgccgacttcaagaggagattcaccttctctctggacacctccaagagcaccgcttatctgcagatgaactctctgagggccgaggataccgccgtctactactgcgccaagtaccctcactactacggcagcagccactggtacttcgatgtgtggggccaaggcactctggtcactgtcagcagcgccagcactaagggccctagcgtcttccctctggcccctagcagcaagagcaccagcggaggaactgctgctctgggctgtctggtgaaggactacttccccgagcccgtgaccgtgagctggaacagcggcgctctgactagcggcgtgcacactttccccgccgtgctgcagagcagcggactgtactctctgagcagcgtggtgactgtccccagcagctctctgggcactcagacctacatctgcaacgtcaaccacaagcccagcaacaccaaggtcgacaagaaggtcgagcctaagagctgc

SEQ ID NO: 44 - DNA, 345 bp, Artificial Sequence
  Nucleotide sequence of Anti-PD-L1 nanobody
gaggtccagctgcaagagagcggcggaggactggtgcaacccggcggctctctgagactcagctgtgccgccagcggcttcaccttcagcagctactggatgtactggctcagacaagcccccggcaaaggactggaatgggtgtccagcatcaacagcgacagcagcagcacctactatagggatagcgtcaagggaaggttcaccatctctagggacaacgccaagaacactctgtatctgcagatgaactctctgaagagcgaggataccgccgtgtactactgcgccaaggatcccggcggctatgctaaaggccaaggcactcaagtcactgtgagcagc

SEQ ID NO: 45 - DNA, 1023 bp, Artificial Sequence
  Nucleotide sequence of Peptide #2 of Bi-74-76
gatatccagatgactcagagccctagctctctgagcgctagcgtgggagatagggtgactatcacttgttccgccagccaagatatctccaactacctcaactggtaccagcagaagcccggcaaggctcccaaggtgctgatctacttcacctcctctctgcacagcggcgtgcctagcagattttccggcagcggctccggcaccgatttcactctgactatcagctctctgcagcccgaggatttcgccacctactactgccagcagtactccaccgtgccttggactttcggccaaggcaccaaggtcgagatcaagaggaccgtcgccgcccccagcgtgttcatcttccctcctagcgatgagcagctgaagagcggcactgccagcgtcgtctgtctgctgaacaatttctaccctagggaggccaaggtgcagtggaaggtggataacgctctgcagagcggcaacagccaagagtccgtcaccgagcaagatagcaaagatagcacctacagcctcagcagcactctgactctgtccaaggccgattacgagaagcacaaggtgtacgcttgcgaggtgactcaccaaggactgagcagccccgtgaccaagagcttcaataggggcgagtgtggcggaggcgggagcggaggcggaggctccggagaggtccagctgcaagagagcggcggaggactggtgcaacccggcggctctctgagactcagctgtgccgccagcggcttcaccttcagcagctactggatgtactggctcagacaagcccccggcaaaggactggaatgggtgtccagcatcaacagcgacagcagcagcacctactatagggatagcgtcaagggaaggttcaccatctctagggacaacgccaagaacactctgtatctgcagatgaactctctgaagagcgaggataccgccgtgtactactgcgccaaggatcccggcggctatgctaaaggccaaggcactcaagtcactgtgagcagctga

SEQ ID NO: 46 - DNA, 321 bp, Artificial Sequence
  Nucleotide sequence of VL chain of anti-VEGF antibody
gatatccagatgactcagagccctagctctctgagcgctagcgtgggagatagggtgactatcacttgttccgccagccaagatatctccaactacctcaactggtaccagcagaagcccggcaaggctcccaaggtgctgatctacttcacctcctctctgcacagcggcgtgcctagcagattttccggcagcggctccggcaccgatttcactctgactatcagctctctgcagcccgaggatttcgccacctactactgccagcagtactccaccgtgccttggactttcggccaaggcaccaaggtcgagatcaag

SEQ ID NO: 47 - DNA, 1032 bp, Artificial Sequence
  Nucleotide sequence of Peptide #1 of Bi-78-79, Bi-79-83, Bi-79-86
gaggtccagctgcaagagagcggcggaggactggtgcaacccggcggctctctgagactcagctgtgccgccagcggcttcaccttcagcagctactggatgtactggctcagacaagcccccggcaaaggactggaatgggtgtccagcatcaacagcgacagcagcagcacctactatagggatagcgtcaagggaaggttcaccatctctagggacaacgccaagaacactctgtatctgcagatgaactctctgaagagcgaggataccgccgtgtactactgcgccaaggatcccggcggctatgctaaaggccaaggcactcaagtcactgtgagcagcgccagcactaagggccctagcgtcttccctctggcccctagcagcaagagcaccagcggaggaactgctgctctgggctgtctggtgaaggactacttccccgagcccgtgaccgtgagctggaacagcggcgctctgactagcggcgtgcacactttccccgccgtgctgcagagcagcggactgtactctctgagcagcgtggtgactgtccccagcagctctctgggcactcagacctacatctgcaacgtcaaccacaagcccagcaacaccaaggtcgacaagaaggtcgagcctaagagctgcggcggaggcgggagcggaggcggaggctccggagaggtgcagctggtcgaaagcggcggcggactggtgcaacccggcaattctctgaggctgagctgtgccgctagcggcttcaccttcagcagcttcggcatgagctgggtcagacaagcccccggcaagggactggagtgggtgagctccatcagcggcagcggaagcgatactctgtacgccgacagcgtgaagggaaggttcaccatctctagggacaacgccaagaccactctgtatctgcagatgaactctctgaggcccgaggataccgccgtgtactactgcaccatcggcggatctctgagcagaagcagccaaggcactctggtcaccgtcagcagc

SEQ ID NO: 48 - DNA, 672 bp, Artificial Sequence
  Nucleotide sequence of Peptide #2 of Bi-78-79, Bi-79-80
caagtgcagctgcaagagagcggaggaggactggtgcaagctggagactctctgaggctgagctgtatcggctctaggaggaccttcactatggcttggtttaggcaagcccccggcaaggagagggagttcgtcgccggcatttggggacccgccgatcataccatctacgccaacagcgtgaagggcagattcgcttgctctagggatgacagcaccaacaccatctttctgcagatgaactctctggagctggaggataccgctctgtatctgtgtgccgccgccgattccagcggcgatgatttcgagtactggggccaaggcacccaagtgactgtgagcagcaggaccgtcgccgcccccagcgtgttcatcttccctcctagcgatgagcagctgaagagcggcactgccagcgtcgtctgtctgctgaacaatttctaccctagggaggccaaggtgcagtggaaggtggataacgctctgcagagcggcaacagccaagagtccgtcaccgagcaagatagcaaagatagcacctacagcctcagcagcactctgactctgtccaaggccgattacgagaagcacaaggtgtacgcttgcgaggtgactcaccaaggactgagcagccccgtgaccaagagcttcaataggggcgagtgttga

SEQ ID NO: 49 - DNA, 348 bp, Artificial Sequence
  Nucleotide sequence of Anti-PD-L2 nanobody
caagtgcagctgcaagagagcggaggaggactggtgcaagctggagactctctgaggctgagctgtatcggctctaggaggaccttcactatggcttggtttaggcaagcccccggcaaggagagggagttcgtcgccggcatttggggacccgccgatcataccatctacgccaacagcgtgaagggcagattcgcttgctctagggatgacagcaccaacaccatctttctgcagatgaactctctggagctggaggataccgctctgtatctgtgtgccgccgccgattccagcggcgatgatttcgagtactggggccaaggcacccaagtgactgtgagcagc

SEQ ID NO: 50 - DNA, 1017 bp, Artificial Sequence
  Nucleotide sequence of Peptide #1 of Bi-78-80
gaggtccagctgcaagagagcggcggaggactggtgcaacccggcggctctctgagactcagctgtgccgccagcggcttcaccttcagcagctactggatgtactggctcagacaagcccccggcaaaggactggaatgggtgtccagcatcaacagcgacagcagcagcacctactatagggatagcgtcaagggaaggttcaccatctctagggacaacgccaagaacactctgtatctgcagatgaactctctgaagagcgaggataccgccgtgtactactgcgccaaggatcccggcggctatgctaaaggccaaggcactcaagtcactgtgagcagcgccagcactaagggccctagcgtcttccctctggcccctagcagcaagagcaccagcggaggaactgctgctctgggctgtctggtgaaggactacttccccgagcccgtgaccgtgagctggaacagcggcgctctgactagcggcgtgcacactttccccgccgtgctgcagagcagcggactgtactctctgagcagcgtggtgactgtccccagcagctctctgggcactcagacctacatctgcaacgtcaaccacaagcccagcaacaccaaggtcgacaagaaggtcgagcctaagagctgcgataagacccataccgaggtgcagctggtcgaaagcggcggcggactggtgcaacccggcaattctctgaggctgagctgtgccgctagcggcttcaccttcagcagcttcggcatgagctgggtcagacaagcccccggcaagggactggagtgggtgagctccatcagcggcagcggaagcgatactctgtacgccgacagcgtgaagggaaggttcaccatctctagggacaacgccaagaccactctgtatctgcagatgaactctctgaggcccgaggataccgccgtgtactactgcaccatcggcggatctctgagcagaagcagccaaggcactctggtcaccgtcagcagctga

SEQ ID NO: 51 - DNA, 1068 bp, Artificial Sequence
  Nucleotide sequence of Peptide #1 of Bi-81-82
gaggtccagctgcaagagagcggcggaggactggtgcaacccggcggctctctgagactcagctgtgccgccagcggcttcaccttcagcagctactggatgtactggctcagacaagcccccggcaaaggactggaatgggtgtccagcatcaacagcgacagcagcagcacctactatagggatagcgtcaagggaaggttcaccatctctagggacaacgccaagaacactctgtatctgcagatgaactctctgaagagcgaggataccgccgtgtactactgcgccaaggatcccggcggctatgctaaaggccaaggcactcaagtcactgtgagcagcggcggaggcgggagcggaggcggaggctccggagccagcactaagggccctagcgtcttccctctggcccctagcagcaagagcaccagcggaggaactgctgctctgggctgtctggtgaaggactacttccccgagcccgtgaccgtgagctggaacagcggcgctctgactagcggcgtgcacactttccccgccgtgctgcagagcagcggactgtactctctgagcagcgtggtgactgtccccagcagctctctgggcactcagacctacatctgcaacgtcaaccacaagcccagcaacaccaaggtcgacaagaaggtcgagcctaagagctgcggcggaggcgggagcggaggcggaggctccggagaggtgcagctggtcgaaagcggcggcggactggtgcaacccggcaattctctgaggctgagctgtgccgctagcggcttcaccttcagcagcttcggcatgagctgggtcagacaagcccccggcaagggactggagtgggtgagctccatcagcggcagcggaagcgatactctgtacgccgacagcgtgaagggaaggttcaccatctctagggacaacgccaagaccactctgtatctgcagatgaactctctgaggcccgaggataccgccgtgtactactgcaccatcggcggatctctgagcagaagcagccaaggcactctggtcaccgtcagcagctga

SEQ ID NO: 52 - DNA, 705 bp, Artificial Sequence
  Nucleotide sequence of Peptide #2 of Bi-81-82
caagtgcagctgcaagagagcggaggaggactggtgcaagctggagactctctgaggctgagctgtatcggctctaggaggaccttcactatggcttggtttaggcaagcccccggcaaggagagggagttcgtcgccggcatttggggacccgccgatcataccatctacgccaacagcgtgaagggcagattcgcttgctctagggatgacagcaccaacaccatctttctgcagatgaactctctggagctggaggataccgctctgtatctgtgtgccgccgccgattccagcggcgatgatttcgagtactggggccaaggcacccaagtgactgtgagcagcggcggaggcgggagcggaggcggaggctccggaaggaccgtcgccgcccccagcgtgttcatcttccctcctagcgatgagcagctgaagagcggcactgccagcgtcgtctgtctgctgaacaatttctaccctagggaggccaaggtgcagtggaaggtggataacgctctgcagagcggcaacagccaagagtccgtcaccgagcaagatagcaaagatagcacctacagcctcagcagcactctgactctgtccaaggccgattacgagaagcacaaggtgtacgcttgcgaggtgactcaccaaggactgagcagccccgtgaccaagagcttcaataggggcgagtgttga

SEQ ID NO: 53 - DNA, 1062 bp, Artificial Sequence
  Nucleotide sequence of Peptide #2 of Bi-79-83
caagtgcagctgcaagagagcggaggaggactggtgcaagctggagactctctgaggctgagctgtatcggctctaggaggaccttcactatggcttggtttaggcaagcccccggcaaggagagggagttcgtcgccggcatttggggacccgccgatcataccatctacgccaacagcgtgaagggcagattcgcttgctctagggatgacagcaccaacaccatctttctgcagatgaactctctggagctggaggataccgctctgtatctgtgtgccgccgccgattccagcggcgatgatttcgagtactggggccaaggcacccaagtgactgtgagcagcaggaccgtcgccgcccccagcgtgttcatcttccctcctagcgatgagcagctgaagagcggcactgccagcgtcgtctgtctgctgaacaatttctaccctagggaggccaaggtgcagtggaaggtggataacgctctgcagagcggcaacagccaagagtccgtcaccgagcaagatagcaaagatagcacctacagcctcagcagcactctgactctgtccaaggccgattacgagaagcacaaggtgtacgcttgcgaggtgactcaccaaggactgagcagccccgtgaccaagagcttcaataggggcgagtgtggcggaggcgggagcggaggcggaggctccggacaagtgcagctgcaagagagcggaggaggactggtccaagctggaggctctctgagactgagctgcgtggccagcggcagcatcttctccatcggcaccatgggctggtacagacaagcccccggcaagcagagggatctggtggctctggtgaccatcgatggcagcaccaattaccccgatagcgtgaagggaaggttcaccatctctagggacaacgtgaagaacaccgtggatctgcagatgaactctctggagcccgaggataccgccgtgtactactgcaatgccaacattaggaccggctggagcagcgtgaggacttactggggccaaggcacccaagtgactgtgtccagc

SEQ ID NO: 54 - DNA, 672 bp, Artificial Sequence
  Nucleotide sequence of Peptide #2 of Bi-79-86
caagtgcagctggtggaaagcggaggaggcctcgtgcctcccggcgagtctctgagactcagctgcgctgcctccggagccatctttaggatcaacactggcgcttggtacagacaagcccccggcaagcagagagagctggtcgcctctctgaccacttacggcaagactacctatgccgacttcgtgaagggaaggttcaccatctctagggatgacgccaagaacaccgtgtatctgcagatgaactctctgaagcccgaggataccgccatctactattgccacatcggccccgagcctaggtatggctactggggccaaggcacccaagtgactgtgagcagcaggaccgtcgccgcccccagcgtgttcatcttccctcctagcgatgagcagctgaagagcggcactgccagcgtcgtctgtctgctgaacaatttctaccctagggaggccaaggtgcagtggaaggtggataacgctctgcagagcggcaacagccaagagtccgtcaccgagcaagatagcaaagatagcacctacagcctcagcagcactctgactctgtccaaggccgattacgagaagcacaaggtgtacgcttgcgaggtgactcaccaaggactgagcagccccgtgaccaagagcttcaataggggcgagtgttga

SEQ ID NO: 55 - DNA, 348 bp, Artificial Sequence
  Nucleotide sequence of Anti-41BB nanobody
caagtgcagctggtggaaagcggaggaggcctcgtgcctcccggcgagtctctgagactcagctgcgctgcctccggagccatctttaggatcaacactggcgcttggtacagacaagcccccggcaagcagagagagctggtcgcctctctgaccacttacggcaagactacctatgccgacttcgtgaagggaaggttcaccatctctagggatgacgccaagaacaccgtgtatctgcagatgaactctctgaagcccgaggataccgccatctactattgccacatcggccccgagcctaggtatggctactggggccaaggcacccaagtgactgtgagcagc

SEQ ID NO: 56 - DNA, 1359 bp, Artificial Sequence
  Nucleotide sequence of Peptide #1 of Bi-203-204
caagtgcaactcgtggaaagcggaggaggactcgtcaagcccggcggaagcctcagactgagctgtgccgccagcggacacacattcatcatctacgccatcggctggtttaggcaagcccccggcaagggactggagttcgtggccacaatcaactggtccggctccatgacaaactacgccgacagcgtgaagggaaggttcactatcagcagagataacgccaagaacacagtgtatctgcagatgaactccctcaagccagacgatacagctgtgtactactgcgccgcttacgtgggcgctactatcagcacagctcactctaggtacgactattggggacaaggcactctggtcactgtcagcagcgccagcacaaaaggcccttccgtcttccctctcgctccaagctccaaaagcacatccggaggaacagccgctctgggctgtctggtgaaggactatttcccagagccagtgacagtgagctggaatagcggagctctgacaagcggcgtgcatacattcccagctgtgctgcagagcagcggcctctactctctgagctccgtggtcacagtgcctagctcctctctgggaacacagacttacatctgcaacgtcaatcataaaccatccaacactaaggtcgacaagaaggtcgagccaaagagctgcgacaagacacacacatgcccaccttgcccagccccagaggccgctggaggaccaagcgtgtttctgttcccacctaagccaaaggacacactgatgatctctaggactccagaggtgacttgtgtggtcgtggatgtcagccacgaggatccagaggtcaagttcaactggtacgtggatggagtcgaggtgcacaacgctaagactaagcctagggaggagcagtacaacagcacatatagggtcgtgagcgtgctgacagtcctccatcaagactggctcaacggcaaggaatacaagtgcaaggtcagcaacaaagctctgccagccccaatcgagaaaactatctccaaggctaagggccagccaagggagccacaagtgtatacactgccaccatctagggaagagatgactaagaaccaagtgagcctcacatgcctcgtgaagggcttctaccctagcgatattgccgtggaatgggaaagcaacggccagccagagaacaactataagacaacaccaccagtgctggactccgatggatccttctttctgtacagcaagctgactgtcgacaagtctaggtggcagcaaggcaacgtgttcagctgtagcgtcatgcacgaggctctgcacaaccactacacacaaaagtctctgtctctgagccccggc

SEQ ID NO: 57 - DNA, 372 bp, Artificial Sequence
  Nucleotide sequence of Anti-PD-L1 nanobody
caagtgcaactcgtggaaagcggaggaggactcgtcaagcccggcggaagcctcagactgagctgtgccgccagcggacacacattcatcatctacgccatcggctggtttaggcaagcccccggcaagggactggagttcgtggccacaatcaactggtccggctccatgacaaactacgccgacagcgtgaagggaaggttcactatcagcagagataacgccaagaacacagtgtatctgcagatgaactccctcaagccagacgatacagctgtgtactactgcgccgcttacgtgggcgctactatcagcacagctcactctaggtacgactattggggacaaggcactctggtcactgtcagcagc

SEQ ID NO: 58 - DNA, 678 bp, Artificial Sequence
  Nucleotide sequence of LALA mutant Fc of human IgG1
gacaagacacacacatgcccaccttgcccagccccagaggccgctggaggaccaagcgtgtttctgttcccacctaagccaaaggacacactgatgatctctaggactccagaggtgacttgtgtggtcgtggatgtcagccacgaggatccagaggtcaagttcaactggtacgtggatggagtcgaggtgcacaacgctaagactaagcctagggaggagcagtacaacagcacatatagggtcgtgagcgtgctgacagtcctccatcaagactggctcaacggcaaggaatacaagtgcaaggtcagcaacaaagctctgccagccccaatcgagaaaactatctccaaggctaagggccagccaagggagccacaagtgtatacactgccaccatctagggaagagatgactaagaaccaagtgagcctcacatgcctcgtgaagggcttctaccctagcgatattgccgtggaatgggaaagcaacggccagccagagaacaactataagacaacaccaccagtgctggactccgatggatccttctttctgtacagcaagctgactgtcgacaagtctaggtggcagcaaggcaacgtgttcagctgtagcgtcatgcacgaggctctgcacaaccactacacacaaaagtctctgtctctgagccccggc

SEQ ID NO: 59 - DNA, 678 bp, Artificial Sequence
  Nucleotide sequence of Peptide #2 of Bi-203-204
gaagtgcagctggtcgagagcggaggaggactcgtgcagcccggcggcagcctcagactcagctgtgccgccagcggaaggactttcagcagcatgactatcggctggtttaggcaagcccccggcaagggactggagtttgtctccggcatcggctggacatccggactgacagtctatgccgacagcgtgaagggaaggttcactatctctagggacaacgccaagaactccatgtatctgcagatgaactctctgagggctgaagacacagccgtgtactactgcgccgctgattccatgaataggggccagttcgactactggggccaaggcactctggtgactgtctccagcagaacagtggccgccccttccgtcttcatctttcctccaagcgacgagcagctcaaaagcggaactgccagcgtcgtctgtctgctgaacaacttctaccctagagaggccaaggtccagtggaaggtcgacaatgctctgcagtccggcaacagccaagagtccgtgactgagcaagacagcaaggacagcacttattctctgtccagcactctcactctcagcaaggctgactacgagaagcacaaggtctatgcttgtgaggtgactcaccaaggactgtccagcccagtgactaagagcttcaataggggagagtgt

SEQ ID NO: 60 - DNA, 357 bp, Artificial Sequence
  Nucleotide sequence of Anti-PD-L2 nanobody
gaagtgcagctggtcgagagcggaggaggactcgtgcagcccggcggcagcctcagactcagctgtgccgccagcggaaggactttcagcagcatgactatcggctggtttaggcaagcccccggcaagggactggagtttgtctccggcatcggctggacatccggactgacagtctatgccgacagcgtgaagggaaggttcactatctctagggacaacgccaagaactccatgtatctgcagatgaactctctgagggctgaagacacagccgtgtactactgcgccgctgattccatgaataggggccagttcgactactggggccaaggcactctggtgactgtctccagc